European Patent Application EP 4 596 585 A1, published August 6, 2025. Title: CONSTRUCTION OF ENGINEERED EXTRACELLULAR VESICLE AND USE THEREOF. Applicant: BEIJING ECHO PHARMACEUTICAL CO., LTD. Application WO. The sequence listing filed with the application follows.

SEQUENCE LISTING (32 sequences)

SEQ ID NO: 1 - protein, 1896 aa, synthetic construct
MPLPPRSLQVLLLLLLLLLLLPGMWAEAGLPRAGGGSQPPFRTFSASDWGLTHLVVHEQTGEVYVGAVNRIYKLSGNLTLLRAHVTGPVEDNEKCYPPPSVQSCPHGLGSTDNVNKLLLLDYAANRLLACGSASQGICQFLRLDDLFKLGEPHHRKEHYLSSVQEAGSMAGVLIAGPPGQGQAKLFVGTPIDGKSEYFPTLSSRRLMANEEDADMFGFVYQDEFVSSQLKIPSDTLSKFPAFDIYYVYSFRSEQFVYYLTLQLDTQLTSPDAAGEHFFTSKIVRLCVDDPKFYSYVEFPIGCEQAGVEYRLVQDAYLSRPGRALAHQLGLAEDEDVLFTVFAQGQKNRVKPPKESALCLFTLRAIKEKIKERIQSCYRGEGKLSLPWLLNKELGCINSPLQIDDDFCGQDFNQPLGGTVTIEGTPLFVDKDDGLTAVAAYDYRGRTVVFAGTRSGRIRKILVDLSNPGGRPALAYESVVAQEGSPILRDLVLSPNHQYLYAMTEKQVTRVPVESCVQYTSCELCLGSRDPHCGWCVLHSICSRRDACERADEPQRFAADLLQCVQLTVQPRNVSVTMSQVPLVLQAWNVPDLSAGVNCSFEDFTESESVLEDGRIHCRSPSAREVAPITRGQGDQRVVKLYLKSKETGKKFASVDFVFYNCSVHQSCLSCVNGSFPCHWCKYRHVCTHNVADCAFLEGRVNVSEDCPQILPSTQIYVPVGVVKPITLAARNLPQPQSGQRGYECLFHIPGSPARVTALRFNSSSLQCQNSSYSYEGNDVSDLPVNLSVVWNGNFVIDNPQNIQAHLYKCPALRESCGLCLKADPRFECGWCVAERRCSLRHHCAADTPASWMHARHGSSRCTDPKILKLSPETGPRQGGTRLTITGENLGLRFEDVRLGVRVGKVLCSPVESEYISAEQIVCEIGDASSVRAHDALVEVCVRDCSPHYRALSPKRFTFVTPTFYRVSPSRGPLSGGTWIGIEGSHLNAGSDVAVSVGGRPCSFSWRNSREIRCLTPPGQSPGSAPIIININRAQLTNPEVKYNYTEDPTILRIDPEWSINSGGTLLTVTGTNLATVREPRIRAKYGGIERENGCLVYNDTTMVCRAPSVANPVRSPPELGERPDELGFVMDNVRSLLVLNSTSFLYYPDPVLEPLSPTGLLELKPSSPLILKGRNLLPPAPGNSRLNYTVLIGSTPCTLTVSETQLLCEAPNLTGQHKVTVRAGGFEFSPGTLQVYSDSLLTLPAIVGIGGGGGLLLLVIVAVLIAYKRKSRDADRTLKRLQLQMDNLESRVALECKEAFAELQTDIHELTNDLDGAGIPFLDYRTYAMRVLFPGIEDHPVLKEMEVQANVEKSLTLFGQLLTKKHFLLTFIRTLEAQRSFSMRDRGNVASLIMTALQGEMEYATGVLKQLLSDLIEKNLESKNHPKLLLRRTESVAEKMLTNWFTFLLYKFLKECAGEPLFMLYCAIKQQMEKGPIDAITGEARYSLSEDKLIRQQIDYKTLTLNCVNPENENAPEVPVKGLDCDTVTQAKEKLLDAAYKGVPYSQRPKAADMDLEWRQGRMARIILQDEDVTTKIDNDWKRLNTLAHYQVTDGSSVALVPKQTSAYNISNSSTFTKSLSRYESMLRTASSPDSLRSRTPMITPDLESGTKLWHLVKNHDHLDQREGDRGSKMVSEIYLTRLLATKGTLQKFVDDLFETIFSTAHRGSALPLAIKYMFDFLDEQADKHQIHDADVRHTWKSNCLPLRFWVNVIKNPQFVFDIHKNSITDACLSVVAQTFMDSCSTSEHKLGKDSPSNKLLYAKDIPNYKSWVERYYADIAKMPAISDQDMSAYLAEQSRLHLSQFNSMSALHEIYSYITKYKDEILAALEKDEQARRQRLRSKLEQVVDTMALSS

SEQ ID NO: 2 - protein, 454 aa, synthetic construct
DPKILKLSPETGPRQGGTRLTITGENLGLRFEDVRLGVRVGKVLCSPVESEYISAEQIVCEIGDASSVRAHDALVEVCVRDCSPHYRALSPKRFTFVTPTFYRVSPSRGPLSGGTWIGIEGSHLNAGSDVAVSVGGRPCSFSWRNSREIRCLTPPGQSPGSAPIIININRAQLTNPEVKYNYTEDPTILRIDPEWSINSGGTLLTVTGTNLATVREPRIRAKYGGIERENGCLVYNDTTMVCRAPSVANPVRSPPELGERPDELGFVMDNVRSLLVLNSTSFLYYPDPVLEPLSPTGLLELKPSSPLILKGRNLLPPAPGNSRLNYTVLIGSTPCTLTVSETQLLCEAPNLTGQHKVTVRAGGFEFSPGTLQVYSDSLLTLPAIVGIGGGGGLLLLVIVAVLIAYKRKSRDADRTLKRLQLQMDNLESRVALECKEAFAELQTDIHELTNDLDG

SEQ ID NO: 3 - protein, 438 aa, synthetic construct
DPKILKLSPETGPRQGGTRLTITGENLGLRFEDVRLGVRVGKVLCSPVESEYISAEQIVCEIGDASSVRAHDALVEVCVRDCSPHYRALSPKRFTFVTPTFYRVSPSRGPLSGGTWIGIEGSHLNAGSDVAVSVGGRPCSFSWRNSREIRCLTPPGQSPGSAPIIININRAQLTNPEVKYNYTEDPTILRIDPEWSINSGGTLLTVTGTNLATVREPRIRAKYGGIERENGCLVYNDTTMVCRAPSVANPVRSPPELGERPDELGFVMDNVRSLLVLNSTSFLYYPDPVLEPLSPTGLLELKPSSPLILKGRNLLPPAPGNSRLNYTVLIGSTPCTLTVSETQLLCEAPNLTGQHKVTVRAGGFEFSPGTLQVYSDSLLTLPAIVGIGGGGGLLLLVIVAVLIAYKRKSRDADRTLKRLQLQMDNLESRVALECKEAF

SEQ ID NO: 4 - protein, 341 aa, synthetic construct
TPTFYRVSPSRGPLSGGTWIGIEGSHLNAGSDVAVSVGGRPCSFSWRNSREIRCLTPPGQSPGSAPIIININRAQLTNPEVKYNYTEDPTILRIDPEWSINSGGTLLTVTGTNLATVREPRIRAKYGGIERENGCLVYNDTTMVCRAPSVANPVRSPPELGERPDELGFVMDNVRSLLVLNSTSFLYYPDPVLEPLSPTGLLELKPSSPLILKGRNLLPPAPGNSRLNYTVLIGSTPCTLTVSETQLLCEAPNLTGQHKVTVRAGGFEFSPGTLQVYSDSLLTLPAIVGIGGGGGLLLLVIVAVLIAYKRKSRDADRTLKRLQLQMDNLESRVALECKEAF

SEQ ID NO: 5 - protein, 255 aa, synthetic construct
EDPTILRIDPEWSINSGGTLLTVTGTNLATVREPRIRAKYGGIERENGCLVYNDTTMVCRAPSVANPVRSPPELGERPDELGFVMDNVRSLLVLNSTSFLYYPDPVLEPLSPTGLLELKPSSPLILKGRNLLPPAPGNSRLNYTVLIGSTPCTLTVSETQLLCEAPNLTGQHKVTVRAGGFEFSPGTLQVYSDSLLTLPAIVGIGGGGGLLLLVIVAVLIAYKRKSRDADRTLKRLQLQMDNLESRVALECKEAF

SEQ ID NO: 6 - protein, 158 aa, synthetic construct
SFLYYPDPVLEPLSPTGLLELKPSSPLILKGRNLLPPAPGNSRLNYTVLIGSTPCTLTVSETQLLCEAPNLTGQHKVTVRAGGFEFSPGTLQVYSDSLLTLPAIVGIGGGGGLLLLVIVAVLIAYKRKSRDADRTLKRLQLQMDNLESRVALECKEAF

SEQ ID NO: 7 - protein, 1694 aa, synthetic construct
MCHQQLVISWFSLVFLASPLVAMWELEKDVYVVEVDWTPDAPGETVNLTCDTPEEDDITWTSDQRHGVIGSGKTLTITVKEFLDAGQYTCHKGGETLSHSHLLLHKKENGIWSTEILKNFKNKTFLKCEAPNYSGRFTCSWLVQRNMDLKFNIKSSSSSPDSRAVTCGMASLSAEKVTLDQRDYEKYSVSCQEDVTCPTAEETLPIELALEARQQNKYENYSTSFFIRDIIKPDPPKNLQMKPLKNSQVEVSWEYPDSWSTPHSYFSLKFFVRIQRKKEKMKETEEGCNQKGAFLVEKTSTEVQCKGGNVCVQAQDRYYNSSCSKWACVPCRVRSGGSGGGSGGGGSGGGGSGGGSGGRVIPVSGPARCLSQSRNLLKTTDDMVKTAREKLKHYSCTAEDIDHEDITRDQTSTLKTCLPLELHKNESCLATRETSSTTRGSCLPPQKTSLMMTLCLGSIYEDLKMYQTEFQAINAALQNHNHQQIILDKGMLVAIDELMQSLNHNGETLRQKPPVGEADPYRVKMKLCILLHAFSTRVVTINRVMGYLSSAGGGGSGGGGSRVVRVPTATLVRVVGTELVIPCNVSDYDGPSEQNFDWSFSSLGSSFVELASTWEVGFPAQLYQERLQRGEILLRRTANDAVELHIKNVQPSDQGHYKCSTPSTDATVQGNYEDTVQVKVLADSLHVGPSARPPPSLSLREGEPFELRCTAASASPLHTHLALLWEVHRGPARRSVLALTHEGRFHPGLGYEQRYHSGDVRLDTVGSDAYRLSVSRALSADQGSYRCIVSEWIAEQGNWQEIQEKAVEVATVVIQPSVLRAAVPKNVSVAEGKELDLTCNITTDRADDVRPEVTWSFSRMPDSTLPGSRVLARLDRDSLVHSSPHVALSHVDARSYHLLVRDVSKENSGYYYCHVSLWAPGHNRSWHKVAEAVSSPAGVGVTWLEPDYQVYLNASKVPGFADDPTELACRVVDTKSGEANVRFTVSWYYRMNRRSDNVVTSELLAVMDGDWTLKYGERSKQRAQDGDFIFSKEHTDTFNFRIQRTTEEDRGNYYCVVSAWTKQRNNSWVKSKDVFSKPVNIFWALEDSVLVVKARQPKPFFAAGNTFEMTCKVSSKNIKSPRYSVLIMAEKPVGDLSSPNETKYIISLDQDSVVKLENWTDASRVDGVVLEKVQEDEFRYRMYQTQVSDAGLYRCMVTAWSPVRGSLWREAATSLSNPIEIDFQTSGPIFNASVHSDTPSVIRGDLIKLFCIITVEGAALDPDDMAFDVSWFAVHSFGLDKAPVLLSSLDRKGIVTTSRRDWKSDLSLERVSVLEFLLQVHGSEDQDFGNYYCSVTPWVKSPTGSWQKEAEIHSKPVFITVKMDVLNAFKYPLLIGVGLSTVIGLLSCLIGYCSSHWCCKKEVQETRRERRRLMSMEMDGGGGSDYKDHDGDYKDHDIDYKDDDDKGGGGSGGGGSVSKGEELFTGVVPILVELDGDVNGHKFSVSGEGEGDATYGKLTLKFICTTGKLPVPWPTLVTTLTYGVQCFSRYPDHMKQHDFFKSAMPEGYVQERTIFFKDDGNYKTRAEVKFEGDTLVNRIELKGIDFKEDGNILGHKLEYNYNSHNVYIMADKQKNGIKVNFKIRHNIEDGSVQLADHYQQNTPIGDGPVLLPDNHYLSTQSALSKDPNEKRDHMVLLEFVTAAGITLGMDELYK

SEQ ID NO: 8 - protein, 1218 aa, synthetic construct
MCHQQLVISWFSLVFLASPLVAMWELEKDVYVVEVDWTPDAPGETVNLTCDTPEEDDITWTSDQRHGVIGSGKTLTITVKEFLDAGQYTCHKGGETLSHSHLLLHKKENGIWSTEILKNFKNKTFLKCEAPNYSGRFTCSWLVQRNMDLKFNIKSSSSSPDSRAVTCGMASLSAEKVTLDQRDYEKYSVSCQEDVTCPTAEETLPIELALEARQQNKYENYSTSFFIRDIIKPDPPKNLQMKPLKNSQVEVSWEYPDSWSTPHSYFSLKFFVRIQRKKEKMKETEEGCNQKGAFLVEKTSTEVQCKGGNVCVQAQDRYYNSSCSKWACVPCRVRSGGSGGGSGGGGSGGGGSGGGSGGRVIPVSGPARCLSQSRNLLKTTDDMVKTAREKLKHYSCTAEDIDHEDITRDQTSTLKTCLPLELHKNESCLATRETSSTTRGSCLPPQKTSLMMTLCLGSIYEDLKMYQTEFQAINAALQNHNHQQIILDKGMLVAIDELMQSLNHNGETLRQKPPVGEADPYRVKMKLCILLHAFSTRVVTINRVMGYLSSAGGGGSGGGGSLELNLTDSENATCLYAKWQMNFTVRYETTNKTYKTVTISDHGTVTYNGSICGDDQNGPKIAVQFGPGFSWIANFTKAASTYSIDSVSFSYNTGDNTTFPDAEDKGILTVDELLAIRIPLNDLFRCNSLSTLEKNDVVQHYWDVLVQAFVQNGTVSTNEFLCDKDKTSTVAPTIHTTVPSPTTTPTPKEKPEAGTYSVNNGNDTCLLATMGLQLNITQDKVASVININPNTTHSTGSCRSHTALLRLNSSTIKYLDFVFAVKNENRFYLKEVNISMYLVNGSVFSIANNNLSYWDAPLGSSYMCNKEQTVSVSGAFQINTFDLRVQPFNVTQGKYSTAQECSLDDDTILIPIIVGAGLSGLIIVIVIAYVIGRRKSYAGYQTLGGGGSDYKDHDGDYKDHDIDYKDDDDKGGGGSGGGGSVSKGEELFTGVVPILVELDGDVNGHKFSVSGEGEGDATYGKLTLKFICTTGKLPVPWPTLVTTLTYGVQCFSRYPDHMKQHDFFKSAMPEGYVQERTIFFKDDGNYKTRAEVKFEGDTLVNRIELKGIDFKEDGNILGHKLEYNYNSHNVYIMADKQKNGIKVNFKIRHNIEDGSVQLADHYQQNTPIGDGPVLLPDNHYLSTQSALSKDPNEKRDHMVLLEFVTAAGITLGMDELYK

SEQ ID NO: 9 - protein, 466 aa, synthetic construct
PPVITRIQPETGPLGGGIRITILGSNLGVQAGDIQRISVAGRNCSFQPERYSVSTRIVCVIEAAETPFTGGVEVDVFGKLGRSPPNVQFTFQQPKPLSVEPQQGPQAGGTTLTIHGTHLDTGSQEDVRVTLNGVPCKVTKFGAQLQCVTGPQATRGQMLLEVSYGGSPVPNPGIFFTYRENPVLRAFEPLRSFASGGRSINVTGQGFSLIQRFAMVVIAEPLQSWQPPREAESLQPMTVVGTDYVFHNDTKVVFLSPAVPEEPEAYNLTVLIEMDGHRALLRTEAGAFEYVPDPTFENFTGGVKKQVNKLIHARGTNLNKAMTLQEAEAFVGAERCTMKTLTETDLYCEPPEVQPPPKRRQKRDTTHNLPEFIVKFGSREWVLGRVEYDTRVSDVPLSLILPLVIVPMVVVIAVSVYCYWRKSQQAEREYEKIKSQLEGLEESVRDRCKKEFTDLMIEMEDQTNDV

SEQ ID NO: 10 - protein, 450 aa, synthetic construct
NPQITEILTVSGPPEGGTRVTIHGVNLGLDFSEIAHHVQVAGVPCTPLPGEYIIAEQIVCEMGHALVGTTSGPVRLCIGECKPEFMTKSHQQYTFVNPSVLSLNPIRGPESGGTMVTITGHYLGAGSSVAVYLGNQTCEFYGRSMSEIVCVSPPSSNGLGPVPVSVSVDRAHVDSNLQFEYIDDPRVQRIEPEWSIASGHTPLTITGFNLDVIQEPRIRVKFNGKESVNVCKVVNTTTLTCLAPSLTTDYRPGLDTVERPDEFGFVFNNVQSLLIYNDTKFIYYPNPTFELLSPTGVLDQKPGSPIILKGKNLCPPASGGAKLNYTVLIGETPCAVTVSETQLLCEPPNLTGQHKVMVHVGGMVFSPGSVSVISDSLLTLPAIVSIAAGGSLLLIIVIIVLIAYKRKSRENDLTLKRLQMQMDNLESRVALECKEAFAELQTDINELTSD

SEQ ID NO: 11 - protein, 491 aa, synthetic construct
PAPLIHSVEPLTGPVDGGTRVTIRGSNLGQHVQDVLGMVTVAGVPCAVDAQEYEVSSSLVCITGASGEEVAGATAVEVPGRGRGVSEHDFAYQDPKVHSIFPARGPRAGGTRLTLNGSKLLTGRLEDIRVVVGDQPCHLLPEQQSEQLRCETSPRPTPATLPVAVWFGATERRLQRGQFKYTLDPNITSAGPTKSFLSGGREICVRGQNLDVVQTPRIRVTVVSRMLQPSQGLGRRRRVVPETACSLGPSCSSQQFEEPCHVNSSQLITCRTPALPGLPEDPWVRVEFILDNLVFDFATLNPTPFSYEADPTLQPLNPEDPTMPFRHKPGSVFSVEGENLDLAMSKEEVVAMIGDGPCVVKTLTRHHLYCEPPVEQPLPRHHALREAPDSLPEFTVQMGNLRFSLGHVQYDGESPGAFPVAAQVGLGVGTSLLALGVIIIVLMYRRKSKQALRDYKKVQIQLENLESSVRDRCKKEFTDLMTEMTDLTSDL

SEQ ID NO: 12 - protein, 343 aa, synthetic construct
VFYIKSIEPQKVSTLGKSNVIVTGANFTRASNITMILKGTSTCDKDVIQVSHVLNDTHMKFSLPSSRKEMKDVCIQFDGGNCSSVGSLSYIALPHCSLIFPATTWISGGQNITMMGRNFDVIDNLIISHELKGNINVSEYCVATYCGFLAPSLKSSKVRTNVTVKLRVQDTYLDCGTLQYREDPRFTGYRVESEVDTELEVKIQKENDNFNISKKDIEITLFHGENGQLNCSFENITRNQDLTTILCKIKGIKTASTIANSSKKVRVKLGNLELYVEQESVPSTWYFLIVLPVLLVIVIFAAVGVTRHKSKELSRKQSQQLELLESELRKEIRDGFAELQMDK

SEQ ID NO: 13 - protein, 456 aa, synthetic construct
GTCPAPEIHAIEPLSGPLDGGTLLTIRGRNLGRRLSDVAHGVWIGGVACEPLPDRYTVSEEIVCVTGPAPGPLSGVVTVNASKEGKSRDRFSYVLPLVHSLEPTMGPKAGGTRITIHGNDLHVGSELQVLVNDTDPCTELMRTDTSIACTMPEGALPAPVPVCVRFERRGCVHGNLTFWYMQNPVITAISPRRSPVSGGRTITVAGERFHMVQNVSMAVHHIGREPTLCKVLNSTLITCPSPGALSNASAPVDFFINGRAYADEVAVAEELLDPEEAQRGSRFRLDYLPNPQFSTAKREKWIKHHPGEPLTLVIHKEQDSLGLQSHEYRVKIGQVSCDIQIVSDRIIHCSVNESLGAAVGQLPITIQVGNFNQTIATLQLGGSETAIIVSIVICSVLLLLSVVALFVFCTKSRRAERYWQKTLLQMEEMESQIREEIRKGFAELQTDMTDLTKELN

SEQ ID NO: 14 - protein, 7 aa, synthetic construct
SDSLLTL

SEQ ID NO: 15 - skipped

SEQ ID NO: 16 - protein, 968 aa, synthetic construct
MCHQQLVISWFSLVFLASPLVARVQPTESIVRFPNITNLCPFGEVFNATRFASVYAWNRKRISNCVADYSVLYNSASFSTFKCYGVSPTKLNDLCFTNVYADSFVIRGDEVRQIAPGQTGKIADYNYKLPDDFTGCVIAWNSNNLDSKVGGNYNYLYRLFRKSNLKPFERDISTEIYQAGSTPCNGVEGFNCYFPLQSYGFQPTNGVGYQPYRVVVLSFELLHAPATVCGPKKSTNLVKNKCVNFGGGGSGGGGSDPKILKLSPETGPRQGGTRLTITGENLGLRFEDVRLGVRVGKVLCSPVESEYISAEQIVCEIGDASSVRAHDALVEVCVRDCSPHYRALSPKRFTFVTPTFYRVSPSRGPLSGGTWIGIEGSHLNAGSDVAVSVGGRPCSFSWRNSREIRCLTPPGQSPGSAPIIININRAQLTNPEVKYNYTEDPTILRIDPEWSINSGGTLLTVTGTNLATVREPRIRAKYGGIERENGCLVYNDTTMVCRAPSVANPVRSPPELGERPDELGFVMDNVRSLLVLNSTSFLYYPDPVLEPLSPTGLLELKPSSPLILKGRNLLPPAPGNSRLNYTVLIGSTPCTLTVSETQLLCEAPNLTGQHKVTVRAGGFEFSPGTLQVYSDSLLTLPAIVGIGGGGGLLLLVIVAVLIAYKRKSRDADRTLKRLQLQMDNLESRVALECKEAFGGGGSDYKDHDGDYKDHDIDYKDDDDKGGGGSGGGGSVSKGEELFTGVVPILVELDGDVNGHKFSVSGEGEGDATYGKLTLKFICTTGKLPVPWPTLVTTLTYGVQCFSRYPDHMKQHDFFKSAMPEGYVQERTIFFKDDGNYKTRAEVKFEGDTLVNRIELKGIDFKEDGNILGHKLEYNYNSHNVYIMADKQKNGIKVNFKIRHNIEDGSVQLADHYQQNTPIGDGPVLLPDNHYLSTQSALSKDPNEKRDHMVLLEFVTAAGITLGMDELYK

SEQ ID NO: 17 - protein, 1288 aa, synthetic construct
MCHQQLVISWFSLVFLASPLVAMGRLASRPLLLALLSLALCRGRMKIICLALVALLLTAQPAMAEIVLTQSPATLSLSPGERATLSCRASQSVSSYLAWYQQKPGQAPRLLIYDASNRATGIPARFSGSGSGTDFTLTISSLEPEDFAVYYCQQRSNWPPLTFGGGTKVEIKRTVAAPSVFIFPPSDEQLKSGTASVVCLLNNFYPREAKVQWKVDNALQSGNSQESVTEQDSKDSTYSLSSTLTLSKADYEKHKVYACEVTHQGLSSPVTKSFNRGECGGSSGSGSGSTGTSSSGTGTSAGTTGTSASTSGSGSGGGGGSGGGGSAGGTATAGASSGSQVQLVESGGGVVQPGRSLRLSCAASGFKFSGYGMHWVRQAPGKGLEWVAVIWYDGSKKYYVDSVKGRFTISRDNSKNTLYLQMNSLRAEDTAVYYCARQMGYWHFDLWGRGTLVTVSSASTKGPSVFPLAPSSKSTSGGTAALGCLVKDYFPEPVTVSWNSGALTSGVHTFPAVLQSSGLYSLSSVVTVPSSSLGTQTYICNVNHKPSNTKVDKKVEPKSCDKTHTGGGGSGGGGSDPKILKLSPETGPRQGGTRLTITGENLGLRFEDVRLGVRVGKVLCSPVESEYISAEQIVCEIGDASSVRAHDALVEVCVRDCSPHYRALSPKRFTFVTPTFYRVSPSRGPLSGGTWIGIEGSHLNAGSDVAVSVGGRPCSFSWRNSREIRCLTPPGQSPGSAPIIININRAQLTNPEVKYNYTEDPTILRIDPEWSINSGGTLLTVTGTNLATVREPRIRAKYGGIERENGCLVYNDTTMVCRAPSVANPVRSPPELGERPDELGFVMDNVRSLLVLNSTSFLYYPDPVLEPLSPTGLLELKPSSPLILKGRNLLPPAPGNSRLNYTVLIGSTPCTLTVSETQLLCEAPNLTGQHKVTVRAGGFEFSPGTLQVYSDSLLTLPAIVGIGGGGGLLLLVIVAVLIAYKRKSRDADRTLKRLQLQMDNLESRVALECKEAFGGGGSDYKDHDGDYKDHDIDYKDDDDKGGGGSGGGGSVSKGEELFTGVVPILVELDGDVNGHKFSVSGEGEGDATYGKLTLKFICTTGKLPVPWPTLVTTLTYGVQCFSRYPDHMKQHDFFKSAMPEGYVQERTIFFKDDGNYKTRAEVKFEGDTLVNRIELKGIDFKEDGNILGHKLEYNYNSHNVYIMADKQKNGIKVNFKIRHNIEDGSVQLADHYQQNTPIGDGPVLLPDNHYLSTQSALSKDPNEKRDHMVLLEFVTAAGITLGMDELYK

SEQ ID NO: 18 - protein, 916 aa, synthetic construct
MCHQQLVISWFSLVFLASPLVAVSKGEELFTGVVPILVELDGDVNGHKFSVSGEGEGDATYGKLTLKFICTTGKLPVPWPTLVTTLTYGVQCFSRYPDHMKQHDFFKSAMPEGYVQERTIFFKDDGNYKTRAEVKFEGDTLVNRIELKGIDFKEDGNILGHKLEYNYNSHNVYIMADKQKNGIKVNFKIRHNIEDGSVQLADHYQQNTPIGDGPVLLPDNHYLSTQSALSKDPNEKRDHMVLLEFVTAAGITLGMDELYKGGGGSGGGGSDPKILKLSPETGPRQGGTRLTITGENLGLRFEDVRLGVRVGKVLCSPVESEYISAEQIVCEIGDASSVRAHDALVEVCVRDCSPHYRALSPKRFTFVTPTFYRVSPSRGPLSGGTWIGIEGSHLNAGSDVAVSVGGRPCSFSWRNSREIRCLTPPGQSPGSAPIIININRAQLTNPEVKYNYTEDPTILRIDPEWSINSGGTLLTVTGTNLATVREPRIRAKYGGIERENGCLVYNDTTMVCRAPSVANPVRSPPELGERPDELGFVMDNVRSLLVLNSTSFLYYPDPVLEPLSPTGLLELKPSSPLILKGRNLLPPAPGNSRLNYTVLIGSTPCTLTVSETQLLCEAPNLTGQHKVTVRAGGFEFSPGTLQVYSDSLLTLPAIVGIGGGGGLLLLVIVAVLIAYKRKSRDADRTLKRLQLQMDNLESRVALECKEAFGGGGSDYKDHDGDYKDHDIDYKDDDDKGGGGSGGGGSMVFTLEDFVGDWRQTAGYNLDQVLEQGGVSSLFQNLGVSVTPIQRIVLSGENGLKIDIHVIIPYEGLSGDQMGQIEKIFKVVYPVDDHHFKVILHYGTLVIDGVTPNMIDYFGRPYEGIAVFDGKKITVTGTLWNGNKIIDERLINPDGSLLFRVTINGVTGWRLCERILA

SEQ ID NO: 19 - protein, 180 aa, synthetic construct
VRSLLVLNSTSFLYYPDPVLEPLSPTGLLELKPSSPLILKGRNLLPPAPGNSRLNYTVLIGSTPCTLTVSETQLLCEAPNLTGQHKVIVRAGGFEFSPGTLQVYSDSLLTLPAIVGIGGGGGLLLLVIVAVLIAYKRKSRDADRTLKRLQLQMDNLESRVALECKEAFAELQTDIHELTN

SEQ ID NO: 20 - protein, 180 aa, synthetic construct
VQSLLIYNDTKFIYYPNPTFELLSPTGVLDQKPGSPIILKGKNLCPPASGGAKLNYTVLIGETPCAVTVSETQLLCEPPNLTGQHKVMVHVGGMVFSPGSVSVISDSLLTLPAIVSIAAGGSLLLIIVIIVLIAYKRKSRENDLTLKRLQMQMDNLESRVALECKEAFAELQTDINELTS

SEQ ID NO: 21 - protein, 7 aa, synthetic construct
ADSLLTL

SEQ ID NO: 22 - protein, 7 aa, synthetic construct
SASLLTL

SEQ ID NO: 23 - protein, 7 aa, synthetic construct
SDALLTL

SEQ ID NO: 24 - protein, 7 aa, synthetic construct
SDSALTL

SEQ ID NO: 25 - protein, 7 aa, synthetic construct
SDSLATL

SEQ ID NO: 26 - protein, 7 aa, synthetic construct
SDSLLAL

SEQ ID NO: 27 - protein, 7 aa, synthetic construct
SDSLLTA

SEQ ID NO: 28 - protein, 7 aa, synthetic construct
SESLLTL

SEQ ID NO: 29 - protein, 7 aa, synthetic construct
SDSLITL

SEQ ID NO: 30 - protein, 8 aa, synthetic construct
SDSALLTL

SEQ ID NO: 31 - protein, 9 aa, synthetic construct
SDSAALLTL

SEQ ID NO: 32 - protein, 10 aa, synthetic construct
SDSAAALLTL